European Patent Application EP 4 775 591 A1, published July 15, 2026. Title: 단백질 변이체 및 이를 이용한 L-아미노산 생산 방법. Applicant: 씨제이제일제당 주식회사. The sequence listing filed with the application follows.

SEQUENCE LISTING (25 sequences)

SEQ ID NO: 1 - DNA, 30 bp, synthetic construct
  source 1..30: mol_type = other DNA
tcgagctcggtacccgttccatcgctgagt

SEQ ID NO: 2 - DNA, 32 bp, synthetic construct
  source 1..32: mol_type = other DNA
tggtttttcgaaagtactacctgattattcca

SEQ ID NO: 3 - DNA, 32 bp, synthetic construct
  source 1..32: mol_type = other DNA
tggaataatcaggtagtactttcgaaaaacca

SEQ ID NO: 4 - DNA, 30 bp, synthetic construct
  source 1..30: mol_type = other DNA
agaggatcccctgaggagtacatgcgcgac

SEQ ID NO: 5 - DNA, 5802 bp, synthetic construct
  source 1..5802: mol_type = other DNA
gttcgcttgctgtccataaaaccgcccagtctagctatcgccatgtaagcccactgcaagctacctgctttctctttgcgcttgcgttttcccttgtccagatagcccagtagctgacattcatccggggtcagcaccgtttctgcggactggctttctacgtgttccgcttcctttagcagcccttgcgccctgagtgcttgcggcagcgtgaagctagcttttatcgccattcgccattcaggctgcgcaactgttgggaagggcgatcggtgcgggcctcttcgctattacgccagctggcgaaagggggatgtgctgcaaggcgattaagttgggtaacgccagggttttcccagtcacgacgttgtaaaacgacggccagtgaattcgagctcggtacccggggatcctctagagtcgacctgcaggcatgcaagcttggcgtaatcatggtcatagctgtttcctgtgtgaaattgttatccgctcacaattccacacaacatacgagccggaagcataaagtgtaaagcctggggtgcctaatgagtgagctaactcacattaattgcgttgcgctcactgcccgctttccagtcgggaaacctgtcgtgccagctgcattaatgaatcggccaacgcgcggggagaggcggtttgcgtattgggcgctcttccgcttcctcgctcactgactcgctgcgctcggtcgttcggctgcggcgagcggtatcagctcactcaaaggcggtaatacggttatccacagaatcaggggataacgcaggaaagaacatgtgagcaaaaggccagcaaaaggccaggaaccgtaaaaaggccgcgttgctggcgtttttccataggctccgcccccctgacgagcatcacaaaaatcgacgctcaagtcagaggtggcgaaacccgacaggactataaagataccaggcgtttccccctggaagctccctcgtgcgctctcctgttccgaccctgccgcttaccggatacctgtccgcctttctcccttcgggaagcgtggcgctttctcaatgctcacgctgtaggtatctcagttcggtgtaggtcgttcgctccaagctgggctgtgtgcacgaaccccccgttcagcccgaccgctgcgccttatccggtaactatcgtcttgagtccaacccggtaagacacgacttatcgccactggcagcagccactggtaacaggattagcagagcgaggtatgtaggcggtgctacagagttcttgaagtggtggcctaactacggctacactagaaggacagtatttggtatctgcgctctgctgaagccagttaccttcggaaaaagagttggtagctcttgatccggcaaacaaaccaccgctggtagcggtggtttttttgtttgcaagcagcagattacgcgcagaaaaaaaggatctcaagaagatcctttgatcttttctacggggtctgacgctcagtggaacgaaaactcacgttaagggattttggtcatgagattatcaaaaaggatcttcacctagatccttttggggtgggcgaagaactccagcatgagatccccgcgctggaggatcatccagccctgatagaaacagaagccactggagcacctcaaaaacaccatcatacactaaatcagtaagttggcagcatcacccgacgcactttgcgccgaataaatacctgtgacggaagatcacttcgcagaataaataaatcctggtgtccctgttgataccgggaagccctgggccaacttttggcgaaaatgagacgttgatcggcacgtaagaggttccaactttcaccataatgaaataagatcactaccgggcgtattttttgagttatcgagattttcaggagctgatagaaacagaagccactggagcacctcaaaaacaccatcatacactaaatcagtaagttggcagcatcacccgacgcactttgcgccgaataaatacctgtgacggaagatcacttcgcagaataaataaatcctggtgtccctgttgataccgggaagccctgggccaacttttggcgaaaatgagacgttgatcggcacgtaagaggttccaactttcaccataatgaaataagatcactaccgggcgtattttttgagttatcgagattttcaggagctctttggcatcgtctctcgcctgtcccctcagttcagtaatttcctgcatttgcctgtttccagtcggtagatattccacaaaacagcagggaagcagcgcttttccgctgcataaccctgcttcggggtcattatagcgattttttcggtatatccatcctttttcgcacgatatacaggattttgccaaagggttcgtgtagactttccttggtgtatccaacggcgtcagccgggcaggataggtgaagtaggcccacccgcgagcgggtgttccttcttcactgtcccttattcgcacctggcggtgctcaacgggaatcctgctctgcgaggctggccggctaccgccggcgtaacagatgagggcaagcggatggctgatgaaaccaagccaaccaggaagggcagcccacctatcaaggtgtactgccttccagacgaacgaagagcgattgaggaaaaggcggcggcggccggcatgagcctgtcggcctacctgctggccgtcggccagggctacaaaatcacgggcgtcgtggactatgagcacgtccgcgagggcgtcccggaaaacgattccgaagcccaacctttcatagaaggcggcggtggaatcgaaatctcgtgatggcaggttgggcgtcgcttggtcggtcatttcgaaaaaggttaggaatacggttagccatttgcctgcttttatatagttcatatgggattcacctttatgttgataagaaataaaagaaaatgccaataggatatcggcattttcttttgcgtttttatttgttaactgttaattgtccttgttcaaggatgctgtctttgacaacagatgttttcttgcctttgatgttcagcaggaagctcggcgcaaacgttgattgtttgtctgcgtagaatcctctgtttgtcatatagcttgtaatcacgacattgtttcctttcgcttgaggtacagcgaagtgtgagtaagtaaaggttacatcgttaggcggatcaagatccatttttaacacaaggccagttttgttcagcggcttgtatgggccagttaaagaattagaaacataaccaagcatgtaaatatcgttagacgtaatgccgtcaatcgtcatttttgatccgcgggagtcagtgaacaggtaccatttgccgttcattttaaagacgttcgcgcgttcaatttcatctgttactgtgttagatgcaatcagcggtttcatcacttttttcagtgtgtaatcatcgtttagctcaatcataccgagagcgccgtttgctaactcagccgtgcgttttttatcgctttgcagaagtttttgactttcttgacggaagaatgatgtgcttttgccatagtatgctttgttaaataaagattcttcgccttggtagccatcttcagttccagtgtttgcttcaaatactaagtatttgtggcctttatcttctacgtagtgaggatctctcagcgtatggttgtcgcctgagctgtagttgccttcatcgatgaactgctgtacattttgatacgtttttccgtcaccgtcaaagattgatttataatcctctacaccgttgatgttcaaagagctgtctgatgctgatacgttaacttgtgcagttgtcagtgtttgtttgccgtaatgtttaccggagaaatcagtgtagaataaacggatttttccgtcagatgtaaatgtggctgaacctgaccattcttgtgtttggtcttttaggatagaatcatttgcatcgaatttgtcgctgtctttaaagacgcggccagcgtttttccagctgtcaatagaagtttcgccgactttttgatagaacatgtaaatcgatgtgtcatccgcatttttaggatctccggctaatgcaaagacgatgtggtagccgtgatagtttgcgacagtgccgtcagcgttttgtaatggccagctgtcccaaacgtccaggccttttgcagaagagatatttttaattgtggacgaatcaaattcagaaacttgatatttttcatttttttgctgttcagggatttgcagcatatcatggcgtgtaatatgggaaatgccgtatgtttccttatatggcttttggttcgtttctttcgcaaacgcttgagttgcgcctcctgccagcagtgcggtagtaaaggttaatactgttgcttgttttgcaaactttttgatgttcatcgttcatgtctccttttttatgtactgtgttagcggtctgcttcttccagccctcctgtttgaagatggcaagttagttacgcacaataaaaaaagacctaaaatatgtaaggggtgacgccaaagtatacactttgccctttacacattttaggtcttgcctgctttatcagtaacaaacccgcgcgatttacttttcgacctcattctattagactctcgtttggattgcaactggtctattttcctcttttgtttgatagaaaatcataaaaggatttgcagactacgggcctaaagaactaaaaaatctatctgtttcttttcattctctgtattttttatagtttctgttgcatgggcataaagttgcctttttaatcacaattcagaaaatatcataatatctcatttcactaaataatagtgaacggcaggtatatgtgatgggttaaaaaggatcaccccagagtcccgctcagaagaactcgtcaagaaggcgatagaaggcgatgcgctgcgaatcgggagcggcgataccgtaaagcacgaggaagcggtcagcccattcgccgccaagctcttcagcaatatcacgggtagccaacgctatgtcctgatagcggtccgccacacccagccggccacagtcgatgaatccagaaaagcggccattttccaccatgatattcggcaagcaggcatcgccatgggtcacgacgagatcctcgccgtcgggcatccgcgccttgagcctggcgaacagttcggctggcgcgagcccctgatgctcttcgtccagatcatcctgatcgacaagaccggcttccatccgagtacgtgctcgctcgatgcgatgtttcgcttggtggtcgaatgggcaggtagccggatcaagcgtatgcagccgccgcattgcatcagccatgatggatactttctcggcaggagcaaggtgagatgacaggagatcctgccccggcacttcgcccaatagcagccagtcccttcccgcttcagtgacaacgtcgagacagctgcgcaaggaacgcccgtcgtggccagccacgatagccgcgctgcctcgtcttggagttcattcagggcaccggacaggtcggtcttgacaaaaagaaccgggcgcccctgcgctgacagccggaacacggcggcatcagagcagccgattgtctgttgtgcccagtcatagccgaatagcctctccacccaagcggccggagaacctgcgtgcaatccatcttgttcaatcatgcgaaacgatcctcatcctgtctcttgatcagatcttgatcccctgcgccatcagatccttggcggcaagaaagccatccagtttactttgcagggcttcccaaccttaccagagggcgccccagctggcaattccg

SEQ ID NO: 6 - DNA, 30 bp, synthetic construct
  source 1..30: mol_type = other DNA
agaggagacacaacatgcgagtgttgaagt

SEQ ID NO: 7 - DNA, 30 bp, synthetic construct
  source 1..30: mol_type = other DNA
gtggtttttcgaaagtttactgatgattca

SEQ ID NO: 8 - DNA, 30 bp, synthetic construct
  source 1..30: mol_type = other DNA
ggaataatcaggtagtttaatttgtggatt

SEQ ID NO: 9 - DNA, 30 bp, synthetic construct
  source 1..30: mol_type = other DNA
acttcaacactcgcatgttgtgtctcctct

SEQ ID NO: 10 - DNA, 20 bp, synthetic construct
  source 1..20: mol_type = other DNA
gctgcgaaatctttgtttcc

SEQ ID NO: 11 - DNA, 20 bp, synthetic construct
  source 1..20: mol_type = other DNA
cccaaacacctcccgtttat

SEQ ID NO: 12 - protein, 820 aa, Escherichia coli
MRVLKFGGTSVANAERFLRVADILESNARQGQVATVLSAPAKITNHLVAMIEKTISGQDALPNISDAERIFAELLTGLAAAQPGFPLAQLKTFVDQEFAQIKHVLHGISLLGQCPDSINAALICRGEKMSIAIMAGVLEARGHNVTVIDPVEKLLAVGHYLESTVDIAESTRRIAASRIPADHMVLMAGFTAGNEKGELVVLGRNGSDYSAAVLAACLRADCCEIWTDVDGVYTCDPRQVPDARLLKSMSYQEAMELSYFGAKVLHPRTITPIAQFQIPCLIKNTGNPQAPGTLIGASRDEDELPVKGISNLNNMAMFSVSGPGMKGMVGMAARVFAAMSRARISVVLITQSSSEYSISFCVPQSDCVRAERAMQEEFYLELKEGLLEPLAVTERLAIISVVGDGMRTLRGISAKFFAALARANINIVAIAQGSSERSISVVVNNDDATTGVRVTHQMLFNTDQVIEVFVIGVGGVGGALLEQLKRQQSWLKNKHIDLRVCGVANSKALLTNVHGLNLENWQEELAQAKEPFNLGRLIRLVKEYHLLNPVIVDCTSSQAVADQYADFLREGFHVVTPNKKANTSSMDYYHLLRHAAEKSRRKFLYDTNVGAGLPVIENLQNLLNAGDELMKFSGILSGSLSYIFGKLDEGMSFSEATTLAREMGYTEPDPRDDLSGMDVARKLLILARETGRELELADIEIEPVLPAEFNAEGDVAAFMANLSQLDDLFAARVAKARDEGKVLRYVGNIDEDGACRVKIAEVDGNDPLFKVKNGENALAFYSHYYQPLPLVLRGYGAGNDVTAAGVFADLLRTLSWKLGV

SEQ ID NO: 13 - protein, 310 aa, Escherichia coli
MVKVYAPASSANMSVGFDVLGAAVTPVDGALLGDVVTVEAAETFSLNNLGRFADKLPSEPRENIVYQCWERFCQELGKQIPVAMTLEKNMPIGSGLGSSACSVVAALMAMNEHCGKPLNDTRLLALMGELEGRISGSIHYDNVAPCFLGGMQLMIEENDIISQQVPGFDEWLWVLAYPGIKVSTAEARAILPAQYRRQDCIAHGRHLAGFIHACYSRQPELAAKLMKDVIAEPYRERLLPGFRQARQAVAEIGAVASGISGSGPTLFALCDKPDTAQRVADWLGKNYLQNQEGFVHICRLDTAGARVLEN

SEQ ID NO: 14 - protein, 428 aa, Escherichia coli
MKLYNLKDHNEQVSFAQAVTQGLGKNQGLFFPHDLPEFSLTEIDEMLKLDFVTRSAKILSAFIGDEIPQEILEERVRAAFAFPAPVANVESDVGCLELFHGPTLAFKDFGGRFMAQMLTHIAGDKPVTILTATSGDTGAAVAHAFYGLPNVKVVILYPRGKISPLQEKLFCTLGGNIETVAIDGDFDACQALVKQAFDDEELKVALGLNSANSINISRLLAQICYYFEAVAQLPQEARNQLVVSVPSGNFGDLTAGLLAKSLGLPVKRFIAATNVNDTVPRFLHDGQWSPKATQATLSNAMDVSQPNNWPRVEELFRRKIWQLKELGYAAVDDETTQQTMRELKELGYTSEPHAAVAYRALRDQLNPGEYGLFLGTAHPAKFKESVEAILGETLDLPKELAERADLPLLSHNLPADFAALRKLMMNHQ

SEQ ID NO: 15 - protein, 820 aa, synthetic construct
MRVLKFGGTSVANAERFLRVADILESNARQGQVATVLSAPAKITNHLVAMIEKTISGQDALPNISDAERIFAELLTGLAAAQPGFPLAQLKTFVDQEFAQIKHVLHGISLLGQCPDSINAALICRGEKMSIAIMAGVLEARGHNVTVIDPVEKLLAVGHYLESTVDIAESTRRIAASRIPADHMVLMAGFTAGNEKGELVVLGRNGSDYSAAVLAACLRADCCEIWTDVDGVYTCDPRQVPDARLLKSMSYQEAMELSYFGAKVLHPRTITPIAQFQIPCLIKNTGNPQAPGTLIGASRDEDELPVKGISNLNNMAMFSVSGPGMKGMVGMAARVFAAMSRARISVVLITQPSSEYSISFCVPQSDCVRAERAMQEEFYLELKEGLLEPLAVTERLAIISVVGDGMRTLRGISAKFFAALARANINIVAIAQRSSERSISVVVNNDDATTGVRVTHQMLFNTDQVIEVFVIGVGGVGGALLEQLKRQQSWLKNKHIDLRVCGVANSKALLTNVHGLNLENRQEELAQAKEPFNLGRLIRLVKEYHLLNPVIVDCTSSQAVADQYADFLREGFHVVTPNKKANTSSMDYYHLLRHAAEKSRRKFLYDTNVGAGLPVIENLQNLLNAGDELMKFSGILSGSLSYIFGKLDEGMSFSEATTLAREMGYTEPDPRDDLSGMDVARKLLILARETGRELELADIEIEPVLPAEFNAEGDVAAFMANLSQLDDLFAARVAKARDEGKVLRYVGNIDEDGACRVKIAEVDGNDPLFKVKNGENALAFYSHYYQPLPLVLRGYGAGNDVTAAGVFADLLRTLSWKLGV

SEQ ID NO: 16 - protein, 820 aa, synthetic construct
MRVLKFGGTSVANAERFLRVADILESNARQGQVATVLSAPAKITNHLVAMIEKTISGRDALPNISDAERIFAELLTGLAAAQPGFPLAQLKTFVDQEFAQIKHVLHGISLLGQCPDSINAALICRGEKMSIAIMAGVLEARGHNVTVIDPVEKLLAVGHYLESTVDIAESTRRIAASRIPADHMVLMAGFTAGNEKGELVVLGRNGSDYSAAVLAACLRADCCEIWTDVDGVYTCDPRQVPDARLLKSMSYQEAMELSYFGAKVLHPRTITPIAQFQIPCLIKNTGNPQAPGTLIGASRDEDELPVKGISNLNNMAMFSVSGPGMKGMVGMAARVFAAMSRARISVVLITQPSSEYSISFCVPQSDCVRAERAMQEEFYLELKEGLLEPLAVTERLAIISVVGDGMRTLRGISAKFFAALARANINIVAIAQRSSERSISVVVNNDDATTGVRVTHQMLFNTDQVIEVFVIGVGGVGGALLEQLKRQQSWLKNKHIDLRVCGVANSKALLTNVHGLNLENRQEELAQAKEPFNLGRLIRLVKEYHLLNPVIVDCTSSQAVADQYADFLREGFHVVTPNKKANTSSMDYYHLLRHAAEKSRRKFLYDTNVGAGLPVIENLQNLLNAGDELMKFSGILSGSLSYIFGKLDEGMSFSEATTLAREMGYTEPDPRDDLSGMDVARKLLILARETGRELELADIEIEPVLPAEFDAEGDVAAFMANLSQLDDLFAARVAKARDEGKVLRYVGNIDEDGACRVKIAEVDGNDPLFKVKNGENALAFYSHYYQPLPLVLRGYGAGNDVTAAGVFADLLRTLSWKLGV

SEQ ID NO: 17 - protein, 820 aa, synthetic construct
MRVLKFGGTSVANAERFLRVADILESNARQGQVATVLSAPAKITNHLVAMIEKTISGQDALPNISDAERIFAELLTGLAAAQPGFPLAQLKTFVDQEFAQIKHVLHGISLLGQCPDSINAALICRGEKMSIAIMAGVLEARGHNVTVIDPVEKLLAVGHYLESTVDIAESTRRIAASRIPADHMVLMAGFTAGNEKGELVVLGRNGSDYSAAVLAACLRADCCEIWTDVDGVYTCDPRQVPDARLLKSMSYQEAMELSYFGAKVLHPRTITPIAQFQIPCLIKNTGNPQAPGTLIGASRDEDELPVKGISNLNNMAMFSVSGPGMKGMVGMAARVFAAMSRARISVVLITQPSSEYSISFCVPQSDCVRAERAMQEEFYLELKEGLLEPLAVTERLAIISVVGDGMRTLRGISAKFFAALARANINIVAIAQRSSERSISVVVNNDDATTGVRVTHQMLFNTDQVIEVFVIGVGGVGGALLEQLKRQQSWLKNKHIDLRVCGVANSKALLTNVHGLNLENRQEELAQAKEPFNLGRLIRLVKEYHLLNPVIVDCTSSQAVADQYADFLREGFHVVTPNKKANTSSMDYYHLLRHAAEKSRRKFLYDTNVGAGLPVIENLQNLLNAGDELMKFSGILSGSLSYIFGKLDEGMSFSEATTLAREMGYTEPDPRDDLSGMDVARKLLILARETGRELELADIEIEPVLPAEFDAEGDVAAFMANLSQLDDLFAARVAKARDEGKVLRYVGNIDEDGACRVKIAEVDGNDPLFKVKNGENALAFYSHYYQPLPLVLRGYGAGNDVTAAGVFADLLRTLSWKLGV

SEQ ID NO: 18 - protein, 820 aa, synthetic construct
MRVLKFGGTSVANAERFLRVADILESNARQGQVATVLSAPAKITNHLVAMIEKTISGRDALPNISDAERIFAELLTGLAAAQPGFPLAQLKTFVDQEFAQIKHVLHGISLLGQCPDSINAALICRGEKMSIAIMAGVLEARGHNVTVIDPVEKLLAVGHYLESTVDIAESTRRIAASRIPADHMVLMAGFTAGNEKGELVVLGRNGSDYSAAVLAACLRADCCEIWTDVDGVYTCDPRQVPDARLLKSMSYQEAMELSYFGAKVLHPRTITPIAQFQIPCLIKNTGNPQAPGTLIGASRDEDELPVKGISNLNNMAMFSVSGPGMKGMVGMAARVFAAMSRARISVVLITQPSSEYSISFCVPQSDCVRAERAMQEEFYLELKEGLLEPLAVTERLAIISVVGDGMRTLRGISAKFFAALARANINIVAIAQRSSERSISVVVNNDDATTGVRVTHQMLFNTDQVIEVFVIGVGGVGGALLEQLKRQQSWLKNKHIDLRVCGVANSKALLTNVHGLNLENRQEELAQAKEPFNLGRLIRLVKEYHLLNPVIVDCTSSQAVADQYADFLREGFHVVTPNKKANTSSMDYYHLLRHAAEKSRRKFLYDTNVGAGLPVIENLQNLLNAGDELMKFSGILSGSLSYIFGKLDEGMSFSEATTLAREMGYTEPDPRDDLSGMDVARKLLILARETGRELELADIEIEPVLPAEFDAEGDVAAFMANLSQLDDLFAARVAKARDEGKVLRYVGNIDEDGACRVKIAEVDGNDPLFKVKNGENALAFYSHCYQPLPLVLRGYGAGNDVTAAGVFADLLRTLSWKLGV

SEQ ID NO: 19 - protein, 310 aa, synthetic construct
MVKVYAPASSANMSVGFDVLGAAVTPVDGALLGDVVTVEAAETFSLNNLGRFADKLPSEPRENIVYQCWERFCQELGKQIPVAMTLEKNMPIGSGLGSSACSVVAALMAMNEHCGKPLNDTRLLALMGELEGRISGSIHYDNVAPCFLGGMQLMIEENDIISQQVPGFDEWLWVLAYPGIKVSTAEARAILPAQYRRQDCIAHGRHLAGFIHACYSRQPELAAKLMKDVIAEPYRERLLPGFRQARRAVAEIGAVASGISGSGPTLFALCDKPDTAQRVADWLGKNYLQNQEGFVHICRLDTAGARVLEN

SEQ ID NO: 20 - protein, 428 aa, synthetic construct
MKLYNLKDHNEQVSFAQAVTQGLGKNQGLFFPHDLPEFSLTEIDEMLKLDFVTRSAKILSAFIGDEIPQEILEERVRAAFAFPAPVANVESDVGCLELFHGPTLAFKDFGGRFMAQMLTHIAGDKPVTILTATSGDTGAAVAHAFYGLPNVKVVILYPRGKISPLQEKLFCTLGGNIETVAIDGDFDACQALAKQAFDDEELKVALGLNSANSINISRLLAQICYYFEAVAQLPQEARNQLVVSVPSGNFGDLTAGLLAKSLGLPVKRFIAATNVNDTVPRFLHDGQWSPKATQATLSNAMDVSQPNNWPRVEELFRRKIWQLKELGYAAVDDETTQQTMRELKELGYTSEPHAAVAYRALRDQLNPGEYGLFLGTAHPAKFKESVEAILGETLDLPKELAERADLPLLSHNLPADFAALRKLMMNHQ

SEQ ID NO: 21 - DNA, 31 bp, synthetic construct
  source 1..31: mol_type = other DNA
gtggtttttcgaaagttcagactcctaactt

SEQ ID NO: 22 - DNA, 2463 bp, synthetic construct
  source 1..2463: mol_type = other DNA
atgcgagtgttgaagttcggcggtacatcagtggcaaatgcagaacgttttctgcgtgttgccgatattctggaaagcaatgccaggcaggggcaggtggccaccgtcctctctgcccccgccaaaatcaccaaccacctggtggcgatgattgaaaaaaccattagcggccaggatgctttacccaatatcagcgatgccgaacgtatttttgccgaacttttgacgggactcgccgccgcccagccggggttcccgctggcgcaattgaaaactttcgtcgatcaggaatttgcccaaataaaacatgtcctgcatggcattagtttgttggggcagtgcccggatagcatcaacgctgcgctgatttgccgtggcgagaaaatgtcgatcgccattatggccggcgtgttagaagcgcgtggtcacaacgttaccgttatcgatccggtcgaaaaactgctggcagtggggcattacctcgaatctaccgtcgatattgctgagtccacccgccgtattgcggcaagccgcattccggctgatcacatggtgttgatggcaggtttcaccgccggtaatgaaaaaggcgaactggtggtacttggacgcaacggttccgactactccgcggcggtgctggctgcctgtttacgcgccgattgttgcgagatttggacggacgttgacggggtctatacctgcgacccgcgtcaggtgcccgatgcgaggttgttgaagtcgatgtcctaccaggaagcgatggagctttcctacttcggcgctaaagttcttcacccccgcaccattacccccatcgcccagttccagatcccttgcctgattaaaaataccggaaatcctcaagcaccaggtacgctcattggtgccagtcgtgatgaagacgaattaccggtcaagggcatttccaatctgaataacatggcaatgttcagcgtttccggcccggggatgaaaggaatggtcggcatggcggcgcgcgtctttgccgcgatgtcgcgcgcccgtatttccgtggtgctgattacgcaaccatcttccgaatacagtatcagtttctgcgttccgcaaagcgactgtgtgcgggctgaacgggcaatgcaggaagagttctacctggaactgaaagaaggcttactggagccgctggcggtgacggaacggctggccattatctcggtggtaggtgatggtatgcgcaccttgcgtgggatctcggcgaaattctttgccgcgctggcccgcgccaatatcaacattgtcgccattgctcagagatcttctgaacgctcaatctctgtcgtggtaaataacgatgatgcgaccactggcgtgcgcgttactcatcagatgctgttcaataccgatcaggttatcgaagtgtttgtgattggcgtcggtggcgttggcggtgcgctgctggagcaactgaagcgtcaacaaagctggctgaagaataagcatatcgacttacgtgtctgcggtgttgccaactcgaaggcactgctcaccaatgtgcatggcctaaatctggaaaaccggcaggaagaactggcgcaagccaaagagccgtttaatctcgggcgcttaattcgcctcgtgaaagaatatcatctgctgaacccggtcattgttgactgcacctccagccaggcagtggcggatcaatatgccgacttcttgcgcgaaggtttccacgttgtcacgccgaacaaaaaggccaacacctcgtcgatggattactaccatctgttgcgtcatgcggcggaaaaatcgcggcgtaaattcctctatgacaccaacgttggggctggattaccggttattgagaacctgcaaaatctgctcaatgctggtgatgaattgatgaagttctccggcattctttcaggttcgctttcttatatcttcggcaagttagacgaaggcatgagtttctccgaggcgaccacgctggcgcgggaaatgggttataccgaaccggacccgcgagatgatctttctggtatggatgtggcgcgtaaactattgattctcgctcgtgaaacgggacgtgaactggagctggcggatattgaaattgaacctgtgctgcccgcagagtttaacgccgagggtgatgttgccgcttttatggcgaatctgtcacaactcgacgatctctttgccgcgcgcgtggcgaaggcccgtgatgaaggaaaagttttgcgctatgttggcaatattgatgaagatggtgcctgccgcgtgaagattgccgaagtggatggtaatgatccgctgttcaaagtgaaaaatggcgaaaacgccctggccttctatagccactattatcagccgctgccgttggtactgcgcggatatggtgcgggcaatgacgttacagctgccggtgtctttgccgatctgctacgtaccctctcatggaagttaggagtctga

SEQ ID NO: 23 - DNA, 2463 bp, synthetic construct
  source 1..2463: mol_type = other DNA
atgcgagtgttgaagttcggcggtacatcagtggcaaatgcagaacgttttctgcgtgttgccgatattctggaaagcaatgccaggcaggggcaggtggccaccgtcctctctgcccccgccaaaatcaccaaccacctggtggcgatgattgaaaaaaccattagcggccgggatgctttacccaatatcagcgatgccgaacgtatttttgccgaacttttgacgggactcgccgccgcccagccggggttcccgctggcgcaattgaaaactttcgtcgatcaggaatttgcccaaataaaacatgtcctgcatggcattagtttgttggggcagtgcccggatagcatcaacgctgcgctgatttgccgtggcgagaaaatgtcgatcgccattatggccggcgtgttagaagcgcgtggtcacaacgttaccgttatcgatccggtcgaaaaactgctggcagtggggcattacctcgaatctaccgtcgatattgctgagtccacccgccgtattgcggcaagccgcattccggctgatcacatggtgttgatggcaggtttcaccgccggtaatgaaaaaggcgaactggtggtacttggacgcaacggttccgactactccgcggcggtgctggctgcctgtttacgcgccgattgttgcgagatttggacggacgttgacggggtctatacctgcgacccgcgtcaggtgcccgatgcgaggttgttgaagtcgatgtcctaccaggaagcgatggagctttcctacttcggcgctaaagttcttcacccccgcaccattacccccatcgcccagttccagatcccttgcctgattaaaaataccggaaatcctcaagcaccaggtacgctcattggtgccagtcgtgatgaagacgaattaccggtcaagggcatttccaatctgaataacatggcaatgttcagcgtttccggcccggggatgaaaggaatggtcggcatggcggcgcgcgtctttgccgcgatgtcgcgcgcccgtatttccgtggtgctgattacgcaaccatcttccgaatacagtatcagtttctgcgttccgcaaagcgactgtgtgcgggctgaacgggcaatgcaggaagagttctacctggaactgaaagaaggcttactggagccgctggcggtgacggaacggctggccattatctcggtggtaggtgatggtatgcgcaccttgcgtgggatctcggcgaaattctttgccgcgctggcccgcgccaatatcaacattgtcgccattgctcagagatcttctgaacgctcaatctctgtcgtggtaaataacgatgatgcgaccactggcgtgcgcgttactcatcagatgctgttcaataccgatcaggttatcgaagtgtttgtgattggcgtcggtggcgttggcggtgcgctgctggagcaactgaagcgtcaacaaagctggctgaagaataagcatatcgacttacgtgtctgcggtgttgccaactcgaaggcactgctcaccaatgtgcatggcctaaatctggaaaaccggcaggaagaactggcgcaagccaaagagccgtttaatctcgggcgcttaattcgcctcgtgaaagaatatcatctgctgaacccggtcattgttgactgcacctccagccaggcagtggcggatcaatatgccgacttcttgcgcgaaggtttccacgttgtcacgccgaacaaaaaggccaacacctcgtcgatggattactaccatctgttgcgtcatgcggcggaaaaatcgcggcgtaaattcctctatgacaccaacgttggggctggattaccggttattgagaacctgcaaaatctgctcaatgctggtgatgaattgatgaagttctccggcattctttcaggttcgctttcttatatcttcggcaagttagacgaaggcatgagtttctccgaggcgactactctggcgcgggaaatgggttataccgaaccggatccgcgagatgatctttctggtatggatgtagcgcgtaagctattgattctcgctcgtgaaacgggacgtgaactggagctggcggatattgaaattgaacctgtgctgcccgcagagtttgacgctgagggtgatgttgccgcttttatggcgaatctgtcacagctcgacgatctctttgccgcgcgcgtggcgaaggcccgtgatgaaggaaaggttttgcgctatgttggcaatattgatgaagatggtgcctgccgcgtgaagattgccgaagtggatggtaatgatccgctgttcaaagtgaaaaatggcgaaaacgccctggccttttatagccactattatcagccgctgccgttggtgctgcgcggatatggtgcgggcaatgacgttacagctgccggtgtctttgccgatctgctacgtaccctctcatggaagttaggagtctga

SEQ ID NO: 24 - DNA, 2463 bp, synthetic construct
  source 1..2463: mol_type = other DNA
atgcgagtgttgaagttcggcggtacatcagtggcaaatgcagaacgttttctgcgtgttgccgatattctggaaagcaatgccaggcaggggcaggtggccaccgtcctctctgcccccgccaaaatcaccaaccacctggtggcgatgattgaaaaaaccattagcggccaggatgctttacccaatatcagcgatgccgaacgtatttttgccgaacttttgacgggactcgccgccgcccagccggggttcccgctggcgcaattgaaaactttcgtcgatcaggaatttgcccaaataaaacatgtcctgcatggcattagtttgttggggcagtgcccggatagcatcaacgctgcgctgatttgccgtggcgagaaaatgtcgatcgccattatggccggcgtgttagaagcgcgtggtcacaacgttaccgttatcgatccggtcgaaaaactgctggcagtggggcattacctcgaatctaccgtcgatattgctgagtccacccgccgtattgcggcaagccgcattccggctgatcacatggtgttgatggcaggtttcaccgccggtaatgaaaaaggcgaactggtggtacttggacgcaacggttccgactactccgcggcggtgctggctgcctgtttacgcgccgattgttgcgagatttggacggacgttgacggggtctatacctgcgacccgcgtcaggtgcccgatgcgaggttgttgaagtcgatgtcctaccaggaagcgatggagctttcctacttcggcgctaaagttcttcacccccgcaccattacccccatcgcccagttccagatcccttgcctgattaaaaataccggaaatcctcaagcaccaggtacgctcattggtgccagtcgtgatgaagacgaattaccggtcaagggcatttccaatctgaataacatggcaatgttcagcgtttccggcccggggatgaaaggaatggtcggcatggcggcgcgcgtctttgccgcgatgtcgcgcgcccgtatttccgtggtgctgattacgcaaccatcttccgaatacagtatcagtttctgcgttccgcaaagcgactgtgtgcgggctgaacgggcaatgcaggaagagttctacctggaactgaaagaaggcttactggagccgctggcggtgacggaacggctggccattatctcggtggtaggtgatggtatgcgcaccttgcgtgggatctcggcgaaattctttgccgcgctggcccgcgccaatatcaacattgtcgccattgctcagagatcttctgaacgctcaatctctgtcgtggtaaataacgatgatgcgaccactggcgtgcgcgttactcatcagatgctgttcaataccgatcaggttatcgaagtgtttgtgattggcgtcggtggcgttggcggtgcgctgctggagcaactgaagcgtcaacaaagctggctgaagaataagcatatcgacttacgtgtctgcggtgttgccaactcgaaggcactgctcaccaatgtgcatggcctaaatctggaaaaccggcaggaagaactggcgcaagccaaagagccgtttaatctcgggcgcttaattcgcctcgtgaaagaatatcatctgctgaacccggtcattgttgactgcacctccagccaggcagtggcggatcaatatgccgacttcttgcgcgaaggtttccacgttgtcacgccgaacaaaaaggccaacacctcgtcgatggattactaccatctgttgcgtcatgcggcggaaaaatcgcggcgtaaattcctctatgacaccaacgttggggctggattaccggttattgagaacctgcaaaatctgctcaatgctggtgatgaattgatgaagttctccggcattctttcaggttcgctttcttatatcttcggcaagttagacgaaggcatgagtttctccgaggcgactactctggcgcgggaaatgggttataccgaaccggatccgcgagatgatctttctggtatggatgtagcgcgtaagctattgattctcgctcgtgaaacgggacgtgaactggagctggcggatattgaaattgaacctgtgctgcccgcagagtttgacgctgagggtgatgttgccgcttttatggcgaatctgtcacagctcgacgatctctttgccgcgcgcgtggcgaaggcccgtgatgaaggaaaggttttgcgctatgttggcaatattgatgaagatggtgcctgccgcgtgaagattgccgaagtggatggtaatgatccgctgttcaaagtgaaaaatggcgaaaacgccctggccttttatagccactattatcagccgctgccgttggtgctgcgcggatatggtgcgggcaatgacgttacagctgccggtgtctttgccgatctgctacgtaccctctcatggaagttaggagtctga

SEQ ID NO: 25 - DNA, 2463 bp, synthetic construct
  source 1..2463: mol_type = other DNA
atgcgagtgttgaagttcggcggtacatcagtggcaaatgcagaacgttttctgcgtgttgccgatattctggaaagcaatgccaggcaggggcaggtggccaccgtcctctctgcccccgccaaaatcaccaaccacctggtggcgatgattgaaaaaaccattagcggccgggatgctttacccaatatcagcgatgccgaacgtatttttgccgaacttttgacgggactcgccgccgcccagccggggttcccgctggcgcaattgaaaactttcgtcgatcaggaatttgcccaaataaaacatgtcctgcatggcattagtttgttggggcagtgcccggatagcatcaacgctgcgctgatttgccgtggcgagaaaatgtcgatcgccattatggccggcgtgttagaagcgcgtggtcacaacgttaccgttatcgatccggtcgaaaaactgctggcagtggggcattacctcgaatctaccgtcgatattgctgagtccacccgccgtattgcggcaagccgcattccggctgatcacatggtgttgatggcaggtttcaccgccggtaatgaaaaaggcgaactggtggtacttggacgcaacggttccgactactccgcggcggtgctggctgcctgtttacgcgccgattgttgcgagatttggacggacgttgacggggtctatacctgcgacccgcgtcaggtgcccgatgcgaggttgttgaagtcgatgtcctaccaggaagcgatggagctttcctacttcggcgctaaagttcttcacccccgcaccattacccccatcgcccagttccagatcccttgcctgattaaaaataccggaaatcctcaagcaccaggtacgctcattggtgccagtcgtgatgaagacgaattaccggtcaagggcatttccaatctgaataacatggcaatgttcagcgtttccggcccggggatgaaaggaatggtcggcatggcggcgcgcgtctttgccgcgatgtcgcgcgcccgtatttccgtggtgctgattacgcaaccatcttccgaatacagtatcagtttctgcgttccgcaaagcgactgtgtgcgggctgaacgggcaatgcaggaagagttctacctggaactgaaagaaggcttactggagccgctggcggtgacggaacggctggccattatctcggtggtaggtgatggtatgcgcaccttgcgtgggatctcggcgaaattctttgccgcgctggcccgcgccaatatcaacattgtcgccattgctcagagatcttctgaacgctcaatctctgtcgtggtaaataacgatgatgcgaccactggcgtgcgcgttactcatcagatgctgttcaataccgatcaggttatcgaagtgtttgtgattggcgtcggtggcgttggcggtgcgctgctggagcaactgaagcgtcaacaaagctggctgaagaataagcatatcgacttacgtgtctgcggtgttgccaactcgaaggcactgctcaccaatgtgcatggcctaaatctggaaaaccggcaggaagaactggcgcaagccaaagagccgtttaatctcgggcgcttaattcgcctcgtgaaagaatatcatctgctgaacccggtcattgttgactgcacctccagccaggcagtggcggatcaatatgccgacttcttgcgcgaaggtttccacgttgtcacgccgaacaaaaaggccaacacctcgtcgatggattactaccatctgttgcgtcatgcggcggaaaaatcgcggcgtaaattcctctatgacaccaacgttggggctggattaccggttattgagaacctgcaaaatctgctcaatgctggtgatgaattgatgaagttctccggcattctttcaggttcgctttcttatatcttcggcaagttagacgaaggcatgagtttctccgaggcgactactctggcgcgggaaatgggttataccgaaccggatccgcgagatgatctttctggtatggatgtagcgcgtaagctattgattctcgctcgtgaaacgggacgtgaactggagctggcggatattgaaattgaacctgtgctgcccgcagagtttgacgctgagggtgatgttgccgcttttatggcgaatctgtcacagctcgacgatctctttgccgcgcgcgtggcgaaggcccgtgatgaaggaaaggttttgcgctatgttggcaatattgatgaagatggtgcctgccgcgtgaagattgccgaagtggatggtaatgatccgctgttcaaagtgaaaaatggcgaaaacgccctggccttctatagccactgttatcagccgctgccgttggtactgcgcggatatggtgcgggcaatgacgttacagctgccggtgtctttgctgatctgctacgtaccctctcatggaagttaggagtctga